European Patent Specification EP 3 702 450 B1, published April 10, 2024. Title: Protein. Applicant: DuPont Nutrition Biosciences ApS. The sequence listing filed with the application follows.

SEQUENCE LISTING (35 sequences)

SEQ ID NO: 1 - protein, 305 aa, Fusarium verticillioides
QAADSINKLIKNKGKLYYGTITDPNLLGVAKDTAIIKADFGAVTPENSGKWDATEPSQGKFNFGSFDQVVNFAQQNGLKVRGHTLVWHSQLPQWVKNINDKATLTKVIENHVTQVVGRYKGKIYAWDVVNEIFEWDGTLRKDSHFNNVFGNDDYVGIAFRAARKADPNAKLYINDYSLDSGSASKVTKGMVPSVKKWLSQGVPVDGIGSQTHLDPGAAGQIQGALTALANSGVKEVAITELDIRTAPANDYATVTKACLNVPKCIGITVWGVSDKNSWRKEHDSLLFDANYNPKPAYTAVVNALR

SEQ ID NO: 2 - DNA, 942 bp, Fusarium verticillioides
attcccaccgccatcgagccccgccaggctgccgacagcatcaacaagctgatcaagaacaagggcaagctctactacggaaccatcaccgaccccaacctgctcggcgtcgcaaaggacaccgccatcatcaaggccgactttggcgccgttacccccgagaactcgggcaagtgggacgccaccgagcccagccagggcaagttcaacttcggtagcttcgaccaggttgtcaactttgcccagcagaatggcctcaaggtccgaggtcacactctggtctggcactctcagctccctcagtgggttaagaacatcaacgacaaggctactctgaccaaggtcattgagaaccacgtcacccaagtcgttggacgctacaagggcaagatctacgcctgggacgtcgtcaacgagatcttcgagtgggacggtaccctccgaaaggactctcacttcaacaacgtcttcggcaacgacgactacgttggcattgccttccgcgccgcccgcaaggctgaccccaacgccaagctgtacatcaacgactacagcctcgactccggcagcgcctccaaggtcaccaagggtatggttccctccgtcaagaagtggctcagccagggcgttcccgtcgacggcattggctctcagactcaccttgaccccggtgccgctggccaaatccagggtgctctcactgccctcgccaattctggtgtcaaggaggttgccatcaccgagctcgacatccgcactgcccccgccaacgactacgctaccgtcaccaaggcctgcctcaacgtccccaagtgcattggtatcaccgtctggggtgtctctgacaagaactcttggcgcaaggagcacgacagtcttctgttcgatgctaactacaaccccaagcctgcttacactgctgttgtcaacgctctccgctaa

SEQ ID NO: 3 - protein, 305 aa, Fusarium oxysporum
QASDSINKLIKNKGKLYYGTITDPNLLGVAKDTAIIKADFGAVTPENSGKWDATEPSQGKFNFGSFDQVVNFAQQNGLKVRGHTLVWHSQLPQWVKNINDKATLTKVIENHVTNVVGRYKGKIYAWDVVNEIFDWDGTLRKDSHFNNVFGNDDYVGIAFRAARKADPNAKLYINDYSLDSGSASKVTKGMVPSVKKWLSQGVPVDGIGSQTHLDPGAAGQIQGALTALANSGVKEVAITELDIRTAPANDYATVTKACLNVPKCIGITVWGVSDKNSWRKEHDSLLFDANYNPKAAYTAVVNALR

SEQ ID NO: 4 - DNA, 942 bp, Fusarium oxysporum
attcccaccgccatcgagccccgccaggcctccgacagcatcaacaagctgatcaagaacaagggcaagctctactacggaaccatcaccgaccccaacctgctcggcgtcgcaaaggacactgccatcatcaaggctgactttggcgccgtcacacccgagaactcgggtaagtgggatgccaccgagcccagccagggcaagttcaacttcggcagcttcgaccaggtcgtcaactttgctcagcagaatggcctcaaggtccgaggtcacactctagtctggcactcccagctccctcagtgggttaagaacatcaacgacaaggctactttgaccaaggtcatcgagaaccacgtcaccaacgtcgttggacgctacaagggcaagatctacgcctgggacgtcgttaacgagatcttcgactgggatggtaccctccgaaaggactctcacttcaacaacgtcttcggcaacgacgactacgttggcattgccttccgcgctgcccgcaaggctgaccccaacgccaagctgtacatcaacgactacagcctcgactccggcagcgcctccaaggtcaccaagggcatggttccctctgtcaagaagtggctcagccagggcgtccccgtcgacggtattggttctcagactcaccttgaccccggtgccgctggccaaatccagggtgctctcactgccctcgccaactctggtgtgaaggaggttgccatcaccgagctcgacatccgcactgcccccgccaacgactacgctaccgttaccaaggcctgcctcaacgtccccaagtgcattggtatcaccgtctggggcgtatctgacaagaactcttggcgcaaggagcacgacagccttctgttcgatgctaactacaaccccaaggctgcttacactgctgttgtcaacgctctccgctaa

SEQ ID NO: 5 - protein, 305 aa, Fusarium sp.
QAADSINKLIKNKGKLYYGTITDPNLLGVAKDTAVIKADFGAVTPENSGKWDATEPSQGNFNFGSFDQVVNFAQQNGLKVRGHTLVWHSQLPQWVKNINDKATLTKVIENHVTQVVGRYKGKIYAWDVVNEIFDWDGTLRKDSHFNNVFGNDDYVGIAFRAARKADPNAKLYINDYSLDSASASKVTKGMVPSVKKWLSQGVPVDGIGSQSHLDPGAAGQVQGALTALANSGVKEVAITELDIRTAPANDYATVTKACLNVPKCIGITVWGVSDKNSWRKEHDSLLFDSNYNPKPAYTAVVNALR

SEQ ID NO: 6 - DNA, 942 bp, Fusarium sp.
attcccaccgccatcgagccccgccaggccgccgacagcatcaacaagctgatcaagaacaagggcaagctctactacggaaccatcaccgaccccaacctgctcggcgtcgcaaaggacaccgccgtcatcaaggccgactttggcgccgtcacccccgagaactcgggcaagtgggacgccaccgagcccagccagggcaacttcaacttcggtagcttcgaccaggtcgtcaactttgctcagcagaatggcctcaaggtccgaggtcacactctggtctggcactctcagctccctcagtgggttaagaacatcaacgacaaggctactctgaccaaggtcattgagaaccacgtcacccaagtcgttggacgctacaagggcaagatctacgcctgggacgttgtcaacgagatcttcgactgggacggtaccctccgaaaggattctcacttcaacaacgtcttcggcaacgatgactacgttggcattgccttccgcgccgcccgcaaggctgaccccaacgccaagctgtacatcaacgactacagcctcgactccgccagcgcctccaaggtcaccaagggcatggtcccctccgtcaagaagtggctcagccagggcgttcccgtcgacggcattggctcccagtctcaccttgaccccggtgccgctggccaagtccagggtgctctcactgccctcgccaactctggtgtcaaggaggttgccatcaccgagctcgacatccgcactgcccccgccaacgactacgccaccgtcaccaaggcctgcctaaacgtccccaagtgcattggtatcaccgtctggggtgtctctgacaagaactcttggcgcaaggagcacgacagccttctgttcgactccaactacaaccccaagcctgcttacactgctgttgtcaacgctctccgctaa

SEQ ID NO: 7 - DNA, 987 bp, Artificial Sequence
  Variant GH10 xylanase sequence
atgaagctgtcttctttcctctacaccgcctcgctggtcgcggccattcccaccgccatcgagccccgccaggctgccgacagcatcgacaagctgatcaagaacaagggcaagctctactacggaaccatcaccgacccccccctgctcggcgtcgcaaaggacgtcgccatcatcaaggccgactttggcgccgttacccccgagaactcgggcaagtgggacgccaccgagccccagcagggcaagttcaccttcggtagcttcgaccaggttgtcaactttgcccagcagaatggcctctacgtccgaggtcacactctggtctggcacggccagctccctcagtgggttaagaacatcaacgacaaggctatgctgaccaaggtcattgagaaccacgtcacccaactcgttggacgctacaagggcaagatctacgcctgggacgtcgtcaacgagatcttcgagtgggacggtaccctccgaaaggactctcacttcaaccaggtcttcggcaacgacgactacgttggcattgccttccgcgccgcccgcaaggctgaccccaacgccaagctgtacatcaacgactacagcctcgactcccagagcgcctccaaggtcaccaagggtatggttccctacgtcaagaagtggctcagccagggcgttcccgtcgacggcattggctctcagactcaccttgaccccggtcaggctccccaaatccagggtgctctcactgccctcgccaattctggtgtcaaggaggttgccatcaccgagctcgacatccgcactgcccccgccaacgactacgctaccgtcaccaaggcctgcctcaacgtccccaagtgcattggtatcaccgtctggggtgtctctgacaagaactcttggcgcaaggagcacgacagtcttctgttcgatgctaactacaaccccaagcctgcttactacgctgttgtcaacgctctccgctaa

SEQ ID NO: 8 - DNA, 987 bp, Artificial Sequence
  Variant GH10 xylanase sequence
atgaagctgtcttctttcctctacaccgcctcgctggtcgcggccattcccaccgccatcgagccccgccaggctgccgacagcatcgacaagctgatcaagaacaagggcaagctctactacggaaccatcaccgacccccccctgctcggcgtcgcaaaggacgtcgccatcatcaaggccgactttggcgccgttacccccgagaactcgggcaagtgggacgccaccgagccccagcagggcaagttcaccttcaccagcttcgaccaggttgtcaactttgcccagcagaatggcctctacgtccgaggtcacactctggtctggcactctcagctccctcagtgggttaagaacatcaacgacaaggctatgctgaccaaggtcattgagaaccacgtcacccaactcgttggacgctacaagggcaagatctacgcctgggacgtcgtcaacgagatcttcgagtgggacggtaccctccgaaaggactctcacttcaaccaggtcttcggcaacgacgactacgttggcattgccttccgcgccgcccgcaaggctgaccccaacgccaagctgtacatcaacgactacagcctcgactcccagagcgcctccaaggtcaccaagggtatggttccctacgtcaagaagtggctcagccagggcgttcccgtcgacggcattggctctcagactcaccttgaccccggtcaggctccccaaatccagggtgctctcactgccctcgccaattctggtgtcaaggaggttgccatcaccgagctcgacatccgcactgcccccgccaacgactacgctaccgtcaccaaggcctgcctcaacgtccccaagtgcattggtatcaccgtctggggtgtctctgacaagaactcttggcgcaaggagcacgacagtcttctgttcgatgctaactacaaccccaagcctgcttactacgctgttgtcaacgctctccgctaa

SEQ ID NO: 9 - DNA, 987 bp, Artificial Sequence
  Variant GH10 xylanase sequence
atgaagctgtcttctttcctctacaccgcctcgctggtcgcggccattcccaccgccatcgagccccgccaggctgccgacagcatcgacaagctgatcaagaacaagggcaagctctactacggaaccatcaccgacccccctctgctcggcgtcgcaaaggacgtcgccatcatcaaggccgactttggcgccgttacccccgagaactcgggcaagtgggacgccaccgagcccagccagggcaagttcaacttcggtagcttcgaccaggttgtcaactttgcccagcagaatggcctctacgtccgaggtcacactctggtctggcacggccagctccctcagtgggttaagaacatcaacgacaaggctactctgaccaaggtcattgagaaccacgtcacccaagtcgttggacgctacaagggcaagatctacgcctgggacgtcgtcaacgagatcttcgagtgggacggtaccctccgaaaggactctcacttcaacaacgtcttcggcaacgacgactacgttggcattgccttccgcgccgcccgcaaggctgaccccaacgccaagctgtacatcaacgactacagcctcgactccggcagcgcctccaaggtcaccaagggtatggttccctccgtcaagaagtggctcagccagggcgttcccgtcgacggcattggctctcagactcaccttgaccccggtcaggctggccaaatccagggtgctctcactgccctcgccaattctggtgtcaaggaggttgccatcaccgagctcgacatccgcactgcccccgccaacgactacgctaccgtcaccaaggcctgcctcaacgtccccaagtgcattggtatcaccgtctggggtgtctctgacaagaactcttggcgcaaggagcacgacagtcttctgttcgatgctaactacaaccccaagcctgcttactacgctgttgtcaacgctctccgctaa

SEQ ID NO: 10 - DNA, 987 bp, Artificial Sequence
  Variant GH10 xylanase sequence
atgaagctgtcttctttcctctacaccgcctcgctggtcgcggccattcccaccgccatcgagccccgccaggctgccgacagcatcgacaagctgatcaagaacaagggcaagctctactacggaaccatcaccgaccccaacctgctcggcgtcgcaaaggacgtcgccatcatcaaggccgactttggcgccgttacccccgagaactcgggcaagtgggacgccaccgagccccagcagggcaagttcaccttcaccagcttcgaccaggttgtcaactttgcccagcagaatggcctctacgtccgaggtcacactctggtctggcacggccagctccctcagtgggttaagaacatcaacgacaaggctactctgaccaaggtcattgagaaccacgtcacccaagtcgttggacgctacaagggcaagatctacgcctgggacgtcgtcaacgagatcttcgagtgggacggtaccctccgaaaggactctcacttcaacaacgtcttcggcaacgacgactacgttggcattgccttccgcgccgcccgcaaggctgaccccaacgccaagctgtacatcaacgactacagcctcgactccggcagcgcctccaaggtcaccaagggtatggttccctccgtcaagaagtggctcagccagggcgttcccgtcgacggcattggctctcagactcaccttgaccccggtcaggctggccaaatccagggtgctctcactgccctcgccaattctggtgtcaaggaggttgccatcaccgagctcgacatccgcactgcccccgccaacgactacgctaccgtcaccaaggcctgcctcaacgtccccaagtgcattggtatcaccgtctggggtgtctctgacaagaactcttggcgcaaggagcacgacagtcttctgttcgatgctaactacaaccccaagcctgcttactacgctgttgtcaacgctctccgctaa

SEQ ID NO: 11 - DNA, 987 bp, Artificial Sequence
  Variant GH10 xylanase sequence
atgaagctgtcttctttcctctacaccgcctcgctggtcgcggccattcccaccgccatcgagccccgccaggctgccgacagcatcgacaagctgatcaagaacaagggcaagctctactacggaaccatcaccgacccccccctgctcggcgtcgcaaaggacgtcgccatcatcaaggccgactttggcgccgttacccccgagaactcgggcaagtgggacgccaccgagcccagccagggcaagttcaacttcaccagcttcgaccaggttgtcaactttgcccagcagaatggcctctacgtccgaggtcacactctggtctggcacggccagctccctcagtgggttaagaacatcaacgacaaggctactctgaccaaggtcattgagaaccacgtcacccaagtcgttggacgctacaagggcaagatctacgcctgggacgtcgtcaacgagatcttcgagtgggacggtaccctccgaaaggactctcacttcaacaacgtcttcggcaacgacgactacgttggcattgccttccgcgccgcccgcaaggctgaccccaacgccaagctgtacatcaacgactacagcctcgactccggcagcgcctccaaggtcaccaagggtatggttccctccgtcaagaagtggctcagccagggcgttcccgtcgacggcattggctctcagactcaccttgaccccggtcaggctggccaaatccagggtgctctcactgccctcgccaattctggtgtcaaggaggttgccatcaccgagctcgacatccgcactgcccccgccaacgactacgctaccgtcaccaaggcctgcctcaacgtccccaagtgcattggtatcaccgtctggggtgtctctgacaagaactcttggcgcaaggagcacgacagtcttctgttcgatgctaactacaaccccaagcctgcttactacgctgttgtcaacgctctccgctaa

SEQ ID NO: 12 - DNA, 1039 bp, Artificial Sequence
  Variant GH10 xylanase sequence
atgaagctgtcttctttcctctacaccgcctcgctggtcgcggccattcccaccgccatcgagccccgccaggctgccgacagcatcgacaagctgatcaagaacaagggcaagctctactacggaaccatcaccgacccccccctgctcggcgtcgcaaaggacgtcgccatcatcaaggccgactttggcgccgttacccccgagaactcgggcaagtgggacgccaccgagccccagcagggcaagttcaccttcggtagcttcgaccaggttgtcaactttgcccagcagaatggcctctacgtccgaggtcacactctggtctggcacggccagctccctcagtgggttaagaacatcaacgacaaggctatgctgaccaaggtcattgagaaccacgtcacccaactcgttggacgctacaagggcaagatctacgcctgggtatgttttattcccccagacttcttcgaaatgactttgctaacatgttcaggacgtcgtcaacgagatcttcgagtgggacggtaccctccgaaaggactctcacttcaaccaggtcttcggcaacgacgactacgttggcattgccttccgcgccgcccgcaaggctgaccccaacgccaagctgtacatcaacgactacagcctcgactcccagagcgcctccaaggtcaccaagggtatggttccctacgtcaagaagtggctcagccagggcgttcccgtcgacggcattggctctcagactcaccttgaccccggtcaggctccccaaatccagggtgctctcactgccctcgccaattctggtgtcaaggaggttgccatcaccgagctcgacatccgcactgcccccgccaacgactacgctaccgtcaccaaggcctgcctcaacgtccccaagtgcattggtatcaccgtctggggtgtctctgacaagaactcttggcgcaaggagcacgacagtcttctgttcgatgctaactacaaccccaagcctgcttactacgctgttgtcaacgctctccgctaa

SEQ ID NO: 13 - DNA, 1039 bp, Artificial Sequence
  Variant GH10 xylanase sequence
atgaagctgtcttctttcctctacaccgcctcgctggtcgcggccattcccaccgccatcgagccccgccaggctgccgacagcatcgacaagctgatcaagaacaagggcaagctctactacggaaccatcaccgacccccccctgctcggcgtcgcaaaggacgtcgccatcatcaaggccgactttggcgccgttacccccgagaactcgggcaagtgggacgccaccgagccccagcagggcaagttcaccttcaccagcttcgaccaggttgtcaactttgcccagcagaatggcctctacgtccgaggtcacactctggtctggcactctcagctccctcagtgggttaagaacatcaacgacaaggctatgctgaccaaggtcattgagaaccacgtcacccaactcgttggacgctacaagggcaagatctacgcctgggtatgttttattcccccagacttcttcgaaatgactttgctaacatgttcaggacgtcgtcaacgagatcttcgagtgggacggtaccctccgaaaggactctcacttcaaccaggtcttcggcaacgacgactacgttggcattgccttccgcgccgcccgcaaggctgaccccaacgccaagctgtacatcaacgactacagcctcgactcccagagcgcctccaaggtcaccaagggtatggttccctacgtcaagaagtggctcagccagggcgttcccgtcgacggcattggctctcagactcaccttgaccccggtcaggctccccaaatccagggtgctctcactgccctcgccaattctggtgtcaaggaggttgccatcaccgagctcgacatccgcactgcccccgccaacgactacgctaccgtcaccaaggcctgcctcaacgtccccaagtgcattggtatcaccgtctggggtgtctctgacaagaactcttggcgcaaggagcacgacagtcttctgttcgatgctaactacaaccccaagcctgcttactacgctgttgtcaacgctctccgctaa

SEQ ID NO: 14 - DNA, 1039 bp, Artificial Sequence
  Variant GH10 xylanase sequence
atgaagctgtcttctttcctctacaccgcctcgctggtcgcggccattcccaccgccatcgagccccgccaggctgccgacagcatcgacaagctgatcaagaacaagggcaagctctactacggaaccatcaccgacccccctctgctcggcgtcgcaaaggacgtcgccatcatcaaggccgactttggcgccgttacccccgagaactcgggcaagtgggacgccaccgagcccagccagggcaagttcaacttcggtagcttcgaccaggttgtcaactttgcccagcagaatggcctctacgtccgaggtcacactctggtctggcacggccagctccctcagtgggttaagaacatcaacgacaaggctactctgaccaaggtcattgagaaccacgtcacccaagtcgttggacgctacaagggcaagatctacgcctgggtatgttttattcccccagacttcttcgaaatgactttgctaacatgttcaggacgtcgtcaacgagatcttcgagtgggacggtaccctccgaaaggactctcacttcaacaacgtcttcggcaacgacgactacgttggcattgccttccgcgccgcccgcaaggctgaccccaacgccaagctgtacatcaacgactacagcctcgactccggcagcgcctccaaggtcaccaagggtatggttccctccgtcaagaagtggctcagccagggcgttcccgtcgacggcattggctctcagactcaccttgaccccggtcaggctggccaaatccagggtgctctcactgccctcgccaattctggtgtcaaggaggttgccatcaccgagctcgacatccgcactgcccccgccaacgactacgctaccgtcaccaaggcctgcctcaacgtccccaagtgcattggtatcaccgtctggggtgtctctgacaagaactcttggcgcaaggagcacgacagtcttctgttcgatgctaactacaaccccaagcctgcttactacgctgttgtcaacgctctccgctaa

SEQ ID NO: 15 - DNA, 1039 bp, Artificial Sequence
  Variant GH10 xylanase sequence
atgaagctgtcttctttcctctacaccgcctcgctggtcgcggccattcccaccgccatcgagccccgccaggctgccgacagcatcgacaagctgatcaagaacaagggcaagctctactacggaaccatcaccgaccccaacctgctcggcgtcgcaaaggacgtcgccatcatcaaggccgactttggcgccgttacccccgagaactcgggcaagtgggacgccaccgagccccagcagggcaagttcaccttcaccagcttcgaccaggttgtcaactttgcccagcagaatggcctctacgtccgaggtcacactctggtctggcacggccagctccctcagtgggttaagaacatcaacgacaaggctactctgaccaaggtcattgagaaccacgtcacccaagtcgttggacgctacaagggcaagatctacgcctgggtatgttttattcccccagacttcttcgaaatgactttgctaacatgttcaggacgtcgtcaacgagatcttcgagtgggacggtaccctccgaaaggactctcacttcaacaacgtcttcggcaacgacgactacgttggcattgccttccgcgccgcccgcaaggctgaccccaacgccaagctgtacatcaacgactacagcctcgactccggcagcgcctccaaggtcaccaagggtatggttccctccgtcaagaagtggctcagccagggcgttcccgtcgacggcattggctctcagactcaccttgaccccggtcaggctggccaaatccagggtgctctcactgccctcgccaattctggtgtcaaggaggttgccatcaccgagctcgacatccgcactgcccccgccaacgactacgctaccgtcaccaaggcctgcctcaacgtccccaagtgcattggtatcaccgtctggggtgtctctgacaagaactcttggcgcaaggagcacgacagtcttctgttcgatgctaactacaaccccaagcctgcttactacgctgttgtcaacgctctccgctaa

SEQ ID NO: 16 - DNA, 1039 bp, Artificial Sequence
  Variant GH10 xylanase sequence
atgaagctgtcttctttcctctacaccgcctcgctggtcgcggccattcccaccgccatcgagccccgccaggctgccgacagcatcgacaagctgatcaagaacaagggcaagctctactacggaaccatcaccgacccccccctgctcggcgtcgcaaaggacgtcgccatcatcaaggccgactttggcgccgttacccccgagaactcgggcaagtgggacgccaccgagcccagccagggcaagttcaacttcaccagcttcgaccaggttgtcaactttgcccagcagaatggcctctacgtccgaggtcacactctggtctggcacggccagctccctcagtgggttaagaacatcaacgacaaggctactctgaccaaggtcattgagaaccacgtcacccaagtcgttggacgctacaagggcaagatctacgcctgggtatgttttattcccccagacttcttcgaaatgactttgctaacatgttcaggacgtcgtcaacgagatcttcgagtgggacggtaccctccgaaaggactctcacttcaacaacgtcttcggcaacgacgactacgttggcattgccttccgcgccgcccgcaaggctgaccccaacgccaagctgtacatcaacgactacagcctcgactccggcagcgcctccaaggtcaccaagggtatggttccctccgtcaagaagtggctcagccagggcgttcccgtcgacggcattggctctcagactcaccttgaccccggtcaggctggccaaatccagggtgctctcactgccctcgccaattctggtgtcaaggaggttgccatcaccgagctcgacatccgcactgcccccgccaacgactacgctaccgtcaccaaggcctgcctcaacgtccccaagtgcattggtatcaccgtctggggtgtctctgacaagaactcttggcgcaaggagcacgacagtcttctgttcgatgctaactacaaccccaagcctgcttactacgctgttgtcaacgctctccgctaa

SEQ ID NO: 17 - protein, 305 aa, Artificial Sequence
  Variant GH10 xylanase sequence
QAADSIDKLIKNKGKLYYGTITDPPLLGVAKDVAIIKADFGAVTPENSGKWDATEPQQGKFTFGSFDQVVNFAQQNGLYVRGHTLVWHGQLPQWVKNINDKAMLTKVIENHVTQLVGRYKGKIYAWDVVNEIFEWDGTLRKDSHFNQVFGNDDYVGIAFRAARKADPNAKLYINDYSLDSQSASKVTKGMVPYVKKWLSQGVPVDGIGSQTHLDPGQAPQIQGALTALANSGVKEVAITELDIRTAPANDYATVTKACLNVPKCIGITVWGVSDKNSWRKEHDSLLFDANYNPKPAYYAVVNALR

SEQ ID NO: 18 - protein, 305 aa, Artificial Sequence
  Variant GH10 xylanase sequence
QAADSIDKLIKNKGKLYYGTITDPPLLGVAKDVAIIKADFGAVTPENSGKWDATEPQQGKFTFTSFDQVVNFAQQNGLYVRGHTLVWHSQLPQWVKNINDKAMLTKVIENHVTQLVGRYKGKIYAWDVVNEIFEWDGTLRKDSHFNQVFGNDDYVGIAFRAARKADPNAKLYINDYSLDSQSASKVTKGMVPYVKKWLSQGVPVDGIGSQTHLDPGQAPQIQGALTALANSGVKEVAITELDIRTAPANDYATVTKACLNVPKCIGITVWGVSDKNSWRKEHDSLLFDANYNPKPAYYAVVNALR

SEQ ID NO: 19 - protein, 305 aa, Artificial Sequence
  Variant GH10 xylanase sequence
QAADSIDKLIKNKGKLYYGTITDPPLLGVAKDVAIIKADFGAVTPENSGKWDATEPSQGKFNFGSFDQVVNFAQQNGLYVRGHTLVWHGQLPQWVKNINDKATLTKVIENHVTQVVGRYKGKIYAWDVVNEIFEWDGTLRKDSHFNNVFGNDDYVGIAFRAARKADPNAKLYINDYSLDSGSASKVTKGMVPSVKKWLSQGVPVDGIGSQTHLDPGQAGQIQGALTALANSGVKEVAITELDIRTAPANDYATVTKACLNVPKCIGITVWGVSDKNSWRKEHDSLLFDANYNPKPAYYAVVNALR

SEQ ID NO: 20 - protein, 305 aa, Artificial Sequence
  Variant GH10 xylanase sequence
QAADSIDKLIKNKGKLYYGTITDPNLLGVAKDVAIIKADFGAVTPENSGKWDATEPQQGKFTFTSFDQVVNFAQQNGLYVRGHTLVWHGQLPQWVKNINDKATLTKVIENHVTQVVGRYKGKIYAWDVVNEIFEWDGTLRKDSHFNNVFGNDDYVGIAFRAARKADPNAKLYINDYSLDSGSASKVTKGMVPSVKKWLSQGVPVDGIGSQTHLDPGQAGQIQGALTALANSGVKEVAITELDIRTAPANDYATVTKACLNVPKCIGITVWGVSDKNSWRKEHDSLLFDANYNPKPAYYAVVNALR

SEQ ID NO: 21 - protein, 305 aa, Artificial Sequence
  Variant GH10 xylanase sequence
QAADSIDKLIKNKGKLYYGTITDPPLLGVAKDVAIIKADFGAVTPENSGKWDATEPSQGKFNFTSFDQVVNFAQQNGLYVRGHTLVWHGQLPQWVKNINDKATLTKVIENHVTQVVGRYKGKIYAWDVVNEIFEWDGTLRKDSHFNNVFGNDDYVGIAFRAARKADPNAKLYINDYSLDSGSASKVTKGMVPSVKKWLSQGVPVDGIGSQTHLDPGQAGQIQGALTALANSGVKEVAITELDIRTAPANDYATVTKACLNVPKCIGITVWGVSDKNSWRKEHDSLLFDANYNPKPAYYAVVNALR

SEQ ID NO: 22 - DNA, 27 bp, Artificial Sequence
  Primer 1
caccatgaagctgtcttctttcctcta

SEQ ID NO: 23 - DNA, 27 bp, Artificial Sequence
  Primer 2
tttttagcggagagcgttgacaacagc

SEQ ID NO: 24 - DNA, 1039 bp, Fusarium verticillioides
atgaagctgtcttctttcctctacaccgcctcgctggtcgcggccattcccaccgccatcgagccccgccaggctgccgacagcatcaacaagctgatcaagaacaagggcaagctctactacggaaccatcaccgaccccaacctgctcggcgtcgcaaaggacaccgccatcatcaaggccgactttggcgccgttacccccgagaactcgggcaagtgggacgccaccgagcccagccagggcaagttcaacttcggtagcttcgaccaggttgtcaactttgcccagcagaatggcctcaaggtccgaggtcacactctggtctggcactctcagctccctcagtgggttaagaacatcaacgacaaggctactctgaccaaggtcattgagaaccacgtcacccaagtcgttggacgctacaagggcaagatctacgcctgggtatgttttattcccccagacttcttcgaaatgactttgctaacatgttcaggacgtcgtcaacgagatcttcgagtgggacggtaccctccgaaaggactctcacttcaacaacgtcttcggcaacgacgactacgttggcattgccttccgcgccgcccgcaaggctgaccccaacgccaagctgtacatcaacgactacagcctcgactccggcagcgcctccaaggtcaccaagggtatggttccctccgtcaagaagtggctcagccagggcgttcccgtcgacggcattggctctcagactcaccttgaccccggtgccgctggccaaatccagggtgctctcactgccctcgccaattctggtgtcaaggaggttgccatcaccgagctcgacatccgcactgcccccgccaacgactacgctaccgtcaccaaggcctgcctcaacgtccccaagtgcattggtatcaccgtctggggtgtctctgacaagaactcttggcgcaaggagcacgacagtcttctgttcgatgctaactacaaccccaagcctgcttacactgctgttgtcaacgctctccgctaa

SEQ ID NO: 25 - DNA, 1039 bp, Fusarium verticillioides; identical to SEQ ID NO: 24

SEQ ID NO: 26 - protein, 328 aa, Fusarium verticillioides
MKLSSFLYTASLVAAIPTAIEPRQAADSINKLIKNKGKLYYGTITDPNLLGVAKDTAIIKADFGAVTPENSGKWDATEPSQGKFNFGSFDQVVNFAQQNGLKVRGHTLVWHSQLPQWVKNINDKATLTKVIENHVTQVVGRYKGKIYAWDVVNEIFEWDGTLRKDSHFNNVFGNDDYVGIAFRAARKADPNAKLYINDYSLDSGSASKVTKGMVPSVKKWLSQGVPVDGIGSQTHLDPGAAGQIQGALTALANSGVKEVAITELDIRTAPANDYATVTKACLNVPKCIGITVWGVSDKNSWRKEHDSLLFDANYNPKPAYTAVVNALR

SEQ ID NO: 27 - protein, 313 aa, Fusarium verticillioides
IPTAIEPRQAADSINKLIKNKGKLYYGTITDPNLLGVAKDTAIIKADFGAVTPENSGKWDATEPSQGKFNFGSFDQVVNFAQQNGLKVRGHTLVWHSQLPQWVKNINDKATLTKVIENHVTQVVGRYKGKIYAWDVVNEIFEWDGTLRKDSHFNNVFGNDDYVGIAFRAARKADPNAKLYINDYSLDSGSASKVTKGMVPSVKKWLSQGVPVDGIGSQTHLDPGAAGQIQGALTALANSGVKEVAITELDIRTAPANDYATVTKACLNVPKCIGITVWGVSDKNSWRKEHDSLLFDANYNPKPAYTAVVNALR

SEQ ID NO: 28 - protein, 328 aa, Fusarium oxysporum
MKLSSFLYTASLVAAIPTAIEPRQASDSINKLIKNKGKLYYGTITDPNLLGVAKDTAIIKADFGAVTPENSGKWDATEPSQGKFNFGSFDQVVNFAQQNGLKVRGHTLVWHSQLPQWVKNINDKATLTKVIENHVTNVVGRYKGKIYAWDVVNEIFDWDGTLRKDSHFNNVFGNDDYVGIAFRAARKADPNAKLYINDYSLDSGSASKVTKGMVPSVKKWLSQGVPVDGIGSQTHLDPGAAGQIQGALTALANSGVKEVAITELDIRTAPANDYATVTKACLNVPKCIGITVWGVSDKNSWRKEHDSLLFDANYNPKAAYTAVVNALR

SEQ ID NO: 29 - protein, 313 aa, Fusarium oxysporum
IPTAIEPRQASDSINKLIKNKGKLYYGTITDPNLLGVAKDTAIIKADFGAVTPENSGKWDATEPSQGKFNFGSFDQVVNFAQQNGLKVRGHTLVWHSQLPQWVKNINDKATLTKVIENHVTNVVGRYKGKIYAWDVVNEIFDWDGTLRKDSHFNNVFGNDDYVGIAFRAARKADPNAKLYINDYSLDSGSASKVTKGMVPSVKKWLSQGVPVDGIGSQTHLDPGAAGQIQGALTALANSGVKEVAITELDIRTAPANDYATVTKACLNVPKCIGITVWGVSDKNSWRKEHDSLLFDANYNPKAAYTAVVNALR

SEQ ID NO: 30 - DNA, 1039 bp, Fusarium oxysporum
atgaagctgtcttccttcctctacaccgcctcgctggtcgcggccattcccaccgccatcgagccccgccaggcctccgacagcatcaacaagctgatcaagaacaagggcaagctctactacggaaccatcaccgaccccaacctgctcggcgtcgcaaaggacactgccatcatcaaggctgactttggcgccgtcacacccgagaactcgggtaagtgggatgccaccgagcccagccagggcaagttcaacttcggcagcttcgaccaggtcgtcaactttgctcagcagaatggcctcaaggtccgaggtcacactctagtctggcactcccagctccctcagtgggttaagaacatcaacgacaaggctactttgaccaaggtcatcgagaaccacgtcaccaacgtcgttggacgctacaagggcaagatctacgcctgggtatgttttcttcactcgaacttcttataaatggctttactaacatgttcaggacgtcgttaacgagatcttcgactgggatggtaccctccgaaaggactctcacttcaacaacgtcttcggcaacgacgactacgttggcattgccttccgcgctgcccgcaaggctgaccccaacgccaagctgtacatcaacgactacagcctcgactccggcagcgcctccaaggtcaccaagggcatggttccctctgtcaagaagtggctcagccagggcgtccccgtcgacggtattggttctcagactcaccttgaccccggtgccgctggccaaatccagggtgctctcactgccctcgccaactctggtgtgaaggaggttgccatcaccgagctcgacatccgcactgcccccgccaacgactacgctaccgttaccaaggcctgcctcaacgtccccaagtgcattggtatcaccgtctggggcgtatctgacaagaactcttggcgcaaggagcacgacagccttctgttcgatgctaactacaaccccaaggctgcttacactgctgttgtcaacgctctccgctaa

SEQ ID NO: 31 - DNA, 987 bp, Fusarium oxysporum
atgaagctgtcttccttcctctacaccgcctcgctggtcgcggccattcccaccgccatcgagccccgccaggcctccgacagcatcaacaagctgatcaagaacaagggcaagctctactacggaaccatcaccgaccccaacctgctcggcgtcgcaaaggacactgccatcatcaaggctgactttggcgccgtcacacccgagaactcgggtaagtgggatgccaccgagcccagccagggcaagttcaacttcggcagcttcgaccaggtcgtcaactttgctcagcagaatggcctcaaggtccgaggtcacactctagtctggcactcccagctccctcagtgggttaagaacatcaacgacaaggctactttgaccaaggtcatcgagaaccacgtcaccaacgtcgttggacgctacaagggcaagatctacgcctgggacgtcgttaacgagatcttcgactgggatggtaccctccgaaaggactctcacttcaacaacgtcttcggcaacgacgactacgttggcattgccttccgcgctgcccgcaaggctgaccccaacgccaagctgtacatcaacgactacagcctcgactccggcagcgcctccaaggtcaccaagggcatggttccctctgtcaagaagtggctcagccagggcgtccccgtcgacggtattggttctcagactcaccttgaccccggtgccgctggccaaatccagggtgctctcactgccctcgccaactctggtgtgaaggaggttgccatcaccgagctcgacatccgcactgcccccgccaacgactacgctaccgttaccaaggcctgcctcaacgtccccaagtgcattggtatcaccgtctggggcgtatctgacaagaactcttggcgcaaggagcacgacagccttctgttcgatgctaactacaaccccaaggctgcttacactgctgttgtcaacgctctccgctaa

SEQ ID NO: 32 - DNA, 1039 bp, Fusarium sp.
atgaagctgtcttctttcctctacaccgcctcgctggtcgcggccattcccaccgccatcgagccccgccaggccgccgacagcatcaacaagctgatcaagaacaagggcaagctctactacggaaccatcaccgaccccaacctgctcggcgtcgcaaaggacaccgccgtcatcaaggccgactttggcgccgtcacccccgagaactcgggcaagtgggacgccaccgagcccagccagggcaacttcaacttcggtagcttcgaccaggtcgtcaactttgctcagcagaatggcctcaaggtccgaggtcacactctggtctggcactctcagctccctcagtgggttaagaacatcaacgacaaggctactctgaccaaggtcattgagaaccacgtcacccaagtcgttggacgctacaagggcaagatctacgcctgggtatgttttcttgcctcgaccttctcaaagatgaatttgctaacatgttcaggacgttgtcaacgagatcttcgactgggacggtaccctccgaaaggattctcacttcaacaacgtcttcggcaacgatgactacgttggcattgccttccgcgccgcccgcaaggctgaccccaacgccaagctgtacatcaacgactacagcctcgactccgccagcgcctccaaggtcaccaagggcatggtcccctccgtcaagaagtggctcagccagggcgttcccgtcgacggcattggctcccagtctcaccttgaccccggtgccgctggccaagtccagggtgctctcactgccctcgccaactctggtgtcaaggaggttgccatcaccgagctcgacatccgcactgcccccgccaacgactacgccaccgtcaccaaggcctgcctaaacgtccccaagtgcattggtatcaccgtctggggtgtctctgacaagaactcttggcgcaaggagcacgacagccttctgttcgactccaactacaaccccaagcctgcttacactgctgttgtcaacgctctccgctaa

SEQ ID NO: 33 - DNA, 987 bp, Fusarium sp.
atgaagctgtcttctttcctctacaccgcctcgctggtcgcggccattcccaccgccatcgagccccgccaggccgccgacagcatcaacaagctgatcaagaacaagggcaagctctactacggaaccatcaccgaccccaacctgctcggcgtcgcaaaggacaccgccgtcatcaaggccgactttggcgccgtcacccccgagaactcgggcaagtgggacgccaccgagcccagccagggcaacttcaacttcggtagcttcgaccaggtcgtcaactttgctcagcagaatggcctcaaggtccgaggtcacactctggtctggcactctcagctccctcagtgggttaagaacatcaacgacaaggctactctgaccaaggtcattgagaaccacgtcacccaagtcgttggacgctacaagggcaagatctacgcctgggacgttgtcaacgagatcttcgactgggacggtaccctccgaaaggattctcacttcaacaacgtcttcggcaacgatgactacgttggcattgccttccgcgccgcccgcaaggctgaccccaacgccaagctgtacatcaacgactacagcctcgactccgccagcgcctccaaggtcaccaagggcatggtcccctccgtcaagaagtggctcagccagggcgttcccgtcgacggcattggctcccagtctcaccttgaccccggtgccgctggccaagtccagggtgctctcactgccctcgccaactctggtgtcaaggaggttgccatcaccgagctcgacatccgcactgcccccgccaacgactacgccaccgtcaccaaggcctgcctaaacgtccccaagtgcattggtatcaccgtctggggtgtctctgacaagaactcttggcgcaaggagcacgacagccttctgttcgactccaactacaaccccaagcctgcttacactgctgttgtcaacgctctccgctaa

SEQ ID NO: 34 - DNA, 40 bp, Artificial Sequence
  Primer 1
ccgcggccgcaccatgaagctgtcttccttcctctacacc

SEQ ID NO: 35 - DNA, 37 bp, Artificial Sequence
  Primer 2
ccggcgcgcccttattagcggagagcgttgacaacag